European Patent Application EP 4 806 924 A1, published September 16, 2026. Title: CHIMERIC ANTIGEN RECEPTOR AND APPLICATION THEREOF. Applicant: GUANGZHOU REFORGENE MEDICINE CO., LTD. Application EP. The sequence listing filed with the application follows.

SEQUENCE LISTING (23 sequences)

SEQ ID NO: 1 - DNA, 1602 bp, synthetic construct
  source 1..1602: mol_type = other DNA
atggcactcccagtgactgcacttttgctgccactggcacttttgctccacgctgctagacctgaggtgcaattggtcgaaaccggtggagggatggtgcagcccgaaggatctcttaagttgagttgtgccgcttctggctttacattcaataagaacgccatgaattgggtacgccaggcacccggaaagggattggaatgggtcgctagaatccggaacaagaccaacaattacgcaacgtactacgctgactccgtgaaagcaaggtttaccatttctagggacgatagtcagtccatgctctacctgcagatgaacaatctgaagatcgaagacaccgctatgtactattgcgtcgccggaaacagcttcgcttattggggccagggtacgttggtgacagtctcagcaggtggaggtggctctggaggaggaggttccggtggaggaggctcagatatcgttatgagccagagtccctcttcactggtcgtgtccattggtgaaaaggtgacaatgacatgcaagtcctcacaatctctgctctattctagcaatcagaaaaactacctggcctggtaccagcagaaacctgggcagagtccaaaactcctgatttactgggcctcatcccgagagagcggagtgccagataggttcaccggcagcggcagcggaacagactttaccttgactatcagcagcgtcaaagccgaggatctcgcggtgtattattgccaacaatattacaactatccactgacatttggcgccgggactaagctggaactcaagactacaacacccgcacctagacctcctactcctgctccaaccattgcaagccaacctctctcacttagacctgaagcatgcagacctgctgcaggcggggctgtacatacaagagggttggattttgcgtgtgatatctacatctgggctccactggctggaacctgtggggtgctgctgctgagtttggtcatcacactgtattgtaatcatagaaacagatctggacggagtagactcctgcactcagactacatgaatatgacaccccgacggccaggacctaccagaggacattaccagccatatgcacctccaagagactttgccgcttacagatccggaaggggccgcggaggactgctttacatcttcggacagccttttatgcgacctgtccaaaccacccaagaggaggatgggtgctcatgtcggtttcctgaggaagaagaaggaggctgcgagctgcgagtaggatttagtaggtcagccgatgcccccgcataccagcaaggtcagaatcagctctacaacgagctgaacctggggaggcgggaggagtatgatgtcctcgacggcagacgggggagagatcccgagatgggcggtggcccaagacggggtaatcctcaggagggcctgtataacgagctccaaggggacggtatggcagaggcctacagcgagatcggaatgggtggagaaaggcgccgcggtggggggcatgacggcttgtatcaagggctctctacggcaactggagatacgtacgatgccttgcacatgcaggcccttccacctagg

SEQ ID NO: 2 - protein, 534 aa, synthetic construct
MALPVTALLLPLALLLHAARPEVQLVETGGGMVQPEGSLKLSCAASGFTFNKNAMNWVRQAPGKGLEWVARIRNKTNNYATYYADSVKARFTISRDDSQSMLYLQMNNLKIEDTAMYYCVAGNSFAYWGQGTLVTVSAGGGGSGGGGSGGGGSDIVMSQSPSSLVVSIGEKVTMTCKSSQSLLYSSNQKNYLAWYQQKPGQSPKLLIYWASSRESGVPDRFTGSGSGTDFTLTISSVKAEDLAVYYCQQYYNYPLTFGAGTKLELKTTTPAPRPPTPAPTIASQPLSLRPEACRPAAGGAVHTRGLDFACDIYIWAPLAGTCGVLLLSLVITLYCNHRNRSGRSRLLHSDYMNMTPRRPGPTRGHYQPYAPPRDFAAYRSGRGRGGLLYIFGQPFMRPVQTTQEEDGCSCRFPEEEEGGCELRVGFSRSADAPAYQQGQNQLYNELNLGRREEYDVLDGRRGRDPEMGGGPRRGNPQEGLYNELQGDGMAEAYSEIGMGGERRRGGGHDGLYQGLSTATGDTYDALHMQALPPR

SEQ ID NO: 3 - DNA, 63 bp, synthetic construct
  source 1..63: mol_type = other DNA
atggcactcccagtgactgcacttttgctgccactggcacttttgctccacgctgctagacct

SEQ ID NO: 4 - protein, 21 aa, synthetic construct
MALPVTALLLPLALLLHAARP

SEQ ID NO: 5 - DNA, 735 bp, synthetic construct
  source 1..735: mol_type = other DNA
gaggtgcaattggtcgaaaccggtggagggatggtgcagcccgaaggatctcttaagttgagttgtgccgcttctggctttacattcaataagaacgccatgaattgggtacgccaggcacccggaaagggattggaatgggtcgctagaatccggaacaagaccaacaattacgcaacgtactacgctgactccgtgaaagcaaggtttaccatttctagggacgatagtcagtccatgctctacctgcagatgaacaatctgaagatcgaagacaccgctatgtactattgcgtcgccggaaacagcttcgcttattggggccagggtacgttggtgacagtctcagcaggtggaggtggctctggaggaggaggttccggtggaggaggctcagatatcgttatgagccagagtccctcttcactggtcgtgtccattggtgaaaaggtgacaatgacatgcaagtcctcacaatctctgctctattctagcaatcagaaaaactacctggcctggtaccagcagaaacctgggcagagtccaaaactcctgatttactgggcctcatcccgagagagcggagtgccagataggttcaccggcagcggcagcggaacagactttaccttgactatcagcagcgtcaaagccgaggatctcgcggtgtattattgccaacaatattacaactatccactgacatttggcgccgggactaagctggaactcaag

SEQ ID NO: 6 - protein, 245 aa, synthetic construct
EVQLVETGGGMVQPEGSLKLSCAASGFTFNKNAMNWVRQAPGKGLEWVARIRNKTNNYATYYADSVKARFTISRDDSQSMLYLQMNNLKIEDTAMYYCVAGNSFAYWGQGTLVTVSAGGGGSGGGGSGGGGSDIVMSQSPSSLVVSIGEKVTMTCKSSQSLLYSSNQKNYLAWYQQKPGQSPKLLIYWASSRESGVPDRFTGSGSGTDFTLTISSVKAEDLAVYYCQQYYNYPLTFGAGTKLELK

SEQ ID NO: 7 - DNA, 135 bp, synthetic construct
  source 1..135: mol_type = other DNA
actacaacacccgcacctagacctcctactcctgctccaaccattgcaagccaacctctctcacttagacctgaagcatgcagacctgctgcaggcggggctgtacatacaagagggttggattttgcgtgtgat

SEQ ID NO: 8 - protein, 45 aa, synthetic construct
TTTPAPRPPTPAPTIASQPLSLRPEACRPAAGGAVHTRGLDFACD

SEQ ID NO: 9 - DNA, 84 bp, synthetic construct
  source 1..84: mol_type = other DNA
atctacatctgggctccactggctggaacctgtggggtgctgctgctgagtttggtcatcacactgtattgtaatcatagaaac

SEQ ID NO: 10 - protein, 28 aa, synthetic construct
IYIWAPLAGTCGVLLLSLVITLYCNHRN

SEQ ID NO: 11 - DNA, 123 bp, synthetic construct
  source 1..123: mol_type = other DNA
agatctggacggagtagactcctgcactcagactacatgaatatgacaccccgacggccaggacctaccagaggacattaccagccatatgcacctccaagagactttgccgcttacagatcc

SEQ ID NO: 12 - protein, 41 aa, synthetic construct
RSGRSRLLHSDYMNMTPRRPGPTRGHYQPYAPPRDFAAYRS

SEQ ID NO: 13 - DNA, 126 bp, synthetic construct
  source 1..126: mol_type = other DNA
ggaaggggccgcggaggactgctttacatcttcggacagccttttatgcgacctgtccaaaccacccaagaggaggatgggtgctcatgtcggtttcctgaggaagaagaaggaggctgcgagctg

SEQ ID NO: 14 - protein, 42 aa, synthetic construct
GRGRGGLLYIFGQPFMRPVQTTQEEDGCSCRFPEEEEGGCEL

SEQ ID NO: 15 - DNA, 336 bp, synthetic construct
  source 1..336: mol_type = other DNA
cgagtaggatttagtaggtcagccgatgcccccgcataccagcaaggtcagaatcagctctacaacgagctgaacctggggaggcgggaggagtatgatgtcctcgacggcagacgggggagagatcccgagatgggcggtggcccaagacggggtaatcctcaggagggcctgtataacgagctccaaggggacggtatggcagaggcctacagcgagatcggaatgggtggagaaaggcgccgcggtggggggcatgacggcttgtatcaagggctctctacggcaactggagatacgtacgatgccttgcgaatgcaggcccttccacctagg

SEQ ID NO: 16 - protein, 112 aa, synthetic construct
RVGFSRSADAPAYQQGQNQLYNELNLGRREEYDVLDGRRGRDPEMGGGPRRGNPQEGLYNELQGDGMAEAYSEIGMGGERRRGGGHDGLYQGLSTATGDTYDALHMQALPPR

SEQ ID NO: 17 - protein, 534 aa, synthetic construct
MALPVTALLLPLALLLHAARPEVQLVETGGGMVQPEGSLKLSCAASGFTFNKNAMNWVRQAPGKGLEWVARIRNKTNNYATYYADSVKARFTISRDDSQSMLYLQMNNLKIEDTAMYYCVAGNSFAYWGQGTLVTVSAGGGGSGGGGSGGGGSDIVMSQSPSSLVVSIGEKVTMTCKSSQSLLYSSNQKNYLAWYQQKPGQSPKLLIYWASSRESGVPDRFTGSGSGTDFTLTISSVKAEDLAVYYCQQYYNYPLTFGAGTKLELKTTTPAPRPPTPAPTIASQPLSLRPEACRPAAGGAVHTRGLDFACDIYIWAPLAGTCGVLLLSLVITLYCNHRNRSKRSRLLHSDYMNMTPRRPGPTRKHYQPYAPPRDFAAYRSKRGRKKLLYIFKQPFMRPVQTTQEEDGCSCRFPEEEEGGCELRVGFSRSADAPAYQQGQNQLYNELNLGRREEYDVLDGRRGRDPEMGGGPRRGNPQEGLYNELQGDGMAEAYSEIGMGGERRRGGGHDGLYQGLSTATGDTYDALHMQALPPR

SEQ ID NO: 18 - protein, 534 aa, synthetic construct
MALPVTALLLPLALLLHAARPEVQLVETGGGMVQPEGSLKLSCAASGFTFNKNAMNWVRQAPGKGLEWVARIRNKTNNYATYYADSVKARFTISRDDSQSMLYLQMNNLKIEDTAMYYCVAGNSFAYWGQGTLVTVSAGGGGSGGGGSGGGGSDIVMSQSPSSLVVSIGEKVTMTCKSSQSLLYSSNQKNYLAWYQQKPGQSPKLLIYWASSRESGVPDRFTGSGSGTDFTLTISSVKAEDLAVYYCQQYYNYPLTFGAGTKLELKTTTPAPRPPTPAPTIASQPLSLRPEACRPAAGGAVHTRGLDFACDIYIWAPLAGTCGVLLLSLVITLYCNHRNRSKRSRLLHSDYMNMTPRRPGPTRKHYQPYAPPRDFAAYRSKRGRKKLLYIFKQPFMRPVQTTQEEDGCSCRFPEEEEGGCELRVKFSRSADAPAYQQGQNQLYNELNLGRREEYDVLDKRRGRDPEMGGKPRRKNPQEGLYNELQKDKMAEAYSEIGMKGERRRGKGHDGLYQGLSTATKDTYDALHMQALPPR

SEQ ID NO: 19 - protein, 534 aa, synthetic construct
MALPVTALLLPLALLLHAARPEVQLVETGGGMVQPEGSLKLSCAASGFTFNKNAMNWVRQAPGKGLEWVARIRNKTNNYATYYADSVKARFTISRDDSQSMLYLQMNNLKIEDTAMYYCVAGNSFAYWGQGTLVTVSAGGGGSGGGGSGGGGSDIVMSQSPSSLVVSIGEKVTMTCKSSQSLLYSSNQKNYLAWYQQKPGQSPKLLIYWASSRESGVPDRFTGSGSGTDFTLTISSVKAEDLAVYYCQQYYNYPLTFGAGTKLELKTTTPAPRPPTPAPTIASQPLSLRPEACRPAAGGAVHTRGLDFACDIYIWAPLAGTCGVLLLSLVITLYCNHRNRSRRSRLLHSDYMNMTPRRPGPTRRHYQPYAPPRDFAAYRSRRGRRRLLYIFRQPFMRPVQTTQEEDGCSCRFPEEEEGGCELRVRFSRSADAPAYQQGQNQLYNELNLGRREEYDVLDRRRGRDPEMGGRPRRRNPQEGLYNELQRDRMAEAYSEIGMRGERRRGRGHDGLYQGLSTATRDTYDALHMQALPPR

SEQ ID NO: 20 - protein, 534 aa, synthetic construct
MALPVTALLLPLALLLHAARPEVQLVETGGGMVQPEGSLKLSCAASGFTFNKNAMNWVRQAPGKGLEWVARIRNKTNNYATYYADSVKARFTISRDDSQSMLYLQMNNLKIEDTAMYYCVAGNSFAYWGQGTLVTVSAGGGGSGGGGSGGGGSDIVMSQSPSSLVVSIGEKVTMTCKSSQSLLYSSNQKNYLAWYQQKPGQSPKLLIYWASSRESGVPDRFTGSGSGTDFTLTISSVKAEDLAVYYCQQYYNYPLTFGAGTKLELKTTTPAPRPPTPAPTIASQPLSLRPEACRPAAGGAVHTRGLDFACDIYIWAPLAGTCGVLLLSLVITLYCNHRNRSHRSRLLHSDYMNMTPRRPGPTRHHYQPYAPPRDFAAYRSHRGRHHLLYIFHQPFMRPVQTTQEEDGCSCRFPEEEEGGCELRVHFSRSADAPAYQQGQNQLYNELNLGRREEYDVLDHRRGRDPEMGGHPRRHNPQEGLYNELQHDHMAEAYSEIGMHGERRRGHGHDGLYQGLSTATHDTYDALHMQALPPR

SEQ ID NO: 21 - protein, 534 aa, synthetic construct
MALPVTALLLPLALLLHAARPEVQLVETGGGMVQPEGSLKLSCAASGFTFNKNAMNWVRQAPGKGLEWVARIRNKTNNYATYYADSVKARFTISRDDSQSMLYLQMNNLKIEDTAMYYCVAGNSFAYWGQGTLVTVSAGGGGSGGGGSGGGGSDIVMSQSPSSLVVSIGEKVTMTCKSSQSLLYSSNQKNYLAWYQQKPGQSPKLLIYWASSRESGVPDRFTGSGSGTDFTLTISSVKAEDLAVYYCQQYYNYPLTFGAGTKLELKTTTPAPRPPTPAPTIASQPLSLRPEACRPAAGGAVHTRGLDFACDIYIWAPLAGTCGVLLLSLVITLYCNHRNRSERSRLLHSDYMNMTPRRPGPTREHYQPYAPPRDFAAYRSERGREELLYIFEQPFMRPVQTTQEEDGCSCRFPEEEEGGCELRVEFSRSADAPAYQQGQNQLYNELNLGRREEYDVLDERRGRDPEMGGEPRRENPQEGLYNELQEDEMAEAYSEIGMEGERRRGEGHDGLYQGLSTATEDTYDALHMQALPPR

SEQ ID NO: 22 - protein, 242 aa, synthetic construct
QVQLVQSGAEVKKPGASVKVSCKASGYTFTDYEMHWVRQAPGQGLEWMGALDPKTGDTAYSQKFKGRVTLTADKSTSTAYMELSSLTSEDTAVYYCTRFYSYTYWGQGTLVTVSSGGGGSGGGGSGGGGSDVVMTQSPLSLPVTPGEPASISCRSSQSLVHSNRNTYLHWYLQKPGQSPQLLIYKVSNRFSGVPDRFSGSGSGTDFTLKISRVEAEDVGVYYCSQNTHVPPTFGQGTKLEIK

SEQ ID NO: 23 - protein, 118 aa, synthetic construct
QVQLVESGGGLVQPGGSLRLSCAASGFTFSNYAMSWVRQAPGKGLEWVAAINSGAGSTYYVDSVKGRFTISRDNAKNTLYLQMNSLKPEDTAVYYCVKEVVTGLYDYWGQGTQVTVSS